European Patent Application EP 4 285 938 A1, published December 6, 2023. Title: Pharmaceutical Composition for Treating or Preventing Malignat Breast Cancer. Applicant: Korea Advanced Institute of Science and Technology. The sequence listing filed with the application follows.

SEQUENCE LISTING (1 sequence)

SEQ ID NO: 1 - DNA, 21 bp, Artificial Sequence
  shBCL11A
gcatagacgatggcactgtta